European Patent Application EP 4 706 639 A1, published March 11, 2026. Title: Complement binding fusion protein. Applicant: Invizius Limited. The sequence listing filed with the application follows.

SEQUENCE LISTING (6 sequences)

SEQ ID NO: 1 - protein, 585 aa, Homo sapiens [sequence omitted]

SEQ ID NO: 2 - protein, 80 aa, Streptococcus pneumoniae
  source 1..80: note = amino acids 69-148 of PspC from the TIGR4 strain of Streptococcus pneumonia
SERDKARKEVEEYVKKIVGESYAKSTKKRHTITVALVNELNNIKNEYLNKIVESTSESQLQILMMESRSKVDEAVSKFEK

SEQ ID NO: 3 - protein, 665 aa, synthetic construct
DAHKSEVAHRFKDLGEENFKALVLIAFAQYLQQCPFEDHVKLVNEVTEFAKTCVADESAENCDKSLHTLFGDKLCTVATLRETYGEMADCCAKQEPERNECFLQHKDDNPNLPRLVRPEVDVMCTAFHDNEETFLKKYLYEIARRHPYFYAPELLFFAKRYKAAFTECCQAADKAACLLPKLDELRDEGKASSAKQRLKCASLQKFGERAFKAWAVARLSQRFPKAEFAEVSKLVTDLTKVHTECCHGDLLECADDRADLAKYICENQDSISSKLKECCEKPLLEKSHCIAEVENDEMPADLPSLAADFVESKDVCKNYAEAKDVFLGMFLYEYARRHPDYSVVLLLRLAKTYETTLEKCCAAADPHECYAKVFDEFKPLVEEPQNLIKQNCELFEQLGEYKFQNALLVRYTKKVPQVSTPTLVEVSRNLGKVGSKCCKHPEAKRMPCAEDYLSVVLNQLCVLHEKTPVSDRVTKCCTESLVNRRPCFSALEVDETYVPKEFNAETFTFHADICTLSEKERQIKKQTALVELVKHKPKATKEQLKAVMDDFAAFVEKCCKADDKETCFAEEGKKLVAASQAALGLSERDKARKEVEEYVKKIVGESYAKSTKKRHTITVALVNELNNIKNEYLNKIVESTSESQLQILMMESRSKVDEAVSKFEK

SEQ ID NO: 4 - protein, 61 aa, synthetic construct
  source 1..61: note = FH9
KSCDIPVFMNARTKNDFTWFKLQDTLDYECHDGYESNTGSTTGSIVCGYNGWSDLPICYER

SEQ ID NO: 5 - DNA, 2666 bp, synthetic construct
  source 1..2666: mol_type = other DNA; note = expression unit VDG-PAOX1-variant-aMF-FP1
atcattattagcttactttcataattgcgactggttccaattgacaagcttttgattttaacgacttttaacgacaacttgagaagatcaaaaaacaactaattattcgaagaattccgaaacgatgagattcccatctattttcaccgctgtcttgttcgctgcctcctctgcattggctgcccctgttaacactaccactgaagacgagactgctcaaattccagctgaagcagttatcggttactctgaccttgagggtgatttcgacgtcgctgttttgcctttctctaactccactaacaacggtttgttgttcattaacaccactatcgcttccattgctgctaaggaagagggtgtctctctcgagaagagagatgcacacaaatcagaagttgctcatagattcaaggacctcggagaagagaacttcaaggctcttgtccttatcgctttcgctcaataccttcagcaatgtccttttgaggaccacgttaagttggtgaacgaagttaccgagttcgctaaaacttgcgtagctgacgaatctgctgagaactgtgacaagtcacttcacactctttttggtgacaagctttgtactgtcgctacccttcgtgaaacctacggcgaaatggccgattgctgtgctaagcaggaacctgaaagaaacgaatgtttcttgcagcacaaggacgataaccccaatcttcctcgtttggttcgtcctgaggtcgacgttatgtgcaccgcttttcatgacaacgaagagactttcttaaagaaatacctttacgaaatcgctcgtcgtcacccatacttctacgctccagagctgttgttcttcgcaaagagatataaggctgctttcactgagtgttgccaagctgctgacaaggcagcttgtctattgcctaagcttgacgaattgcgagatgagggtaaagcatcttccgccaagcagagattgaaatgcgcttccttgcagaagtttggtgagcgagctttcaaagcctgggccgtggctaggttgagccaacgttttcctaaagctgagttcgctgaagtttctaagttggttactgatcttactaaggtgcacactgaatgttgccacggtgaccttctggagtgtgctgatgaccgtgcagatttggctaagtatatttgtgaaaaccaagattctatttcttctaaactaaaggaatgttgtgaaaagccacttcttgagaaaagtcactgtatcgctgaggtggagaacgacgagatgccagctgaccttcctagcctggctgctgatttcgttgaatctaaggacgtatgcaagaattacgcagaggccaaggatgttttccttggcatgtttttgtacgagtacgctagaagacaccctgactactccgtagttctcttgctgaggttggcaaagacctacgagactaccctagagaagtgttgcgccgcagctgatcctcacgagtgttatgctaaagtttttgatgagtttaaacctttggttgaggagccacaaaacttgattaagcagaactgcgagcttttcgaacaattgggggaatacaagttccaaaatgccttgctagtcaggtacaccaaaaaggtccctcaggtcagcaccccaaccttagtcgaggtgtccagaaatttgggcaaagttggttctaaatgttgcaagcacccagaagctaagaggatgccatgtgccgaagactacctttccgtcgttctgaaccaactctgtgttttgcacgaaaagactccagtctcagaccgtgtcacgaaatgttgtaccgagtctctggttaacagaagaccttgtttctctgctttggaagttgacgaaacttacgtcccaaaggagttcaacgcggagactttcaccttccacgccgacatttgtacactttccgagaaggaaagacaaatcaagaagcaaaccgcactagttgaattggttaaacataagcctaaggctaccaaagaacaattgaaagcagttatggatgattttgcggctttcgtggaaaagtgttgtaaggctgatgacaaggaaacctgtttcgccgaagaaggtaagaagttagtcgccgcctctcaggctgctcttggactgtccgagagagacaaggctagaaaggaagttgaagagtatgtgaaaaagattgttggtgagtcttacgctaagtctactaaaaagcgtcacactatcaccgtcgcccttgttaacgagttgaataacattaaaaacgaatacctcaacaagatcgtcgaatctacctctgaatctcagctacaaattctgatgatggaatccagatccaaggttgatgaggcagtatcaaagttcgagaagtaatagcggccgctcaagaggatgtcagaatgccatttgcctgagagatgcaggcttcatttttgatacttttttatttgtaacctatatagtataggattttttttgtcattttgtttcttctcgtacgagcttgctcctgatcagcctatctcgcagcagatgaatatcttgtggtaggggtttgggaaaatcattcgagtttgatgtttttcttggtatttcccactcctcttcagagtacagaagattaagtgagaccttcgtttgtgcggatccttcagtaatgtct

SEQ ID NO: 6 - DNA, 1482 bp, synthetic construct
  source 1..1482: mol_type = other DNA; note = expression unit VDG-PAOX1-variant-aMF-FH9-(N529Q)
atcattattagcttactttcataattgcgactggttccaattgacaagcttttgattttaacgacttttaacgacaacttgagaagatcaaaaaacaactaattattcgaagaattccgaaacgatgagattcccatctattttcaccgctgtcttgttcgctgcctcctctgcattggctgcccctgttaacactaccactgaagacgagactgctcaaattccagctgaagcagttatcggttactctgaccttgagggtgatttcgacgtcgctgttttgcctttctctaactccactaacaacggtttgttgttcattaacaccactatcgcttccattgctgctaaggaagagggtgtctctctcgagaagagaaagtcctgcgacatccctgttttcatgaatgctagaactaaaaacgatttcacttggtttaagcttcaagacactctcgattacgagtgtcacgacggttacgaatctaacaccggatcaaccacaggttctattgtctgtggttacaacggttggtctgacctgccaatttgttatgagagataatagcggccgctcaagaggatgtcagaatgccatttgcctgagagatgcaggcttcatttttgatacttttttatttgtaacctatatagtataggattttttttgtcattttgtttcttctcgtacgagcttgctcctgatcagcctatctcgcagcagatgaatatcttgtggtaggggtttgggaaaatcattcgagtttgatgtttttcttggtatttcccactcctcttcagagtacagaagattaagtgagaccttcgtttgtgcggatccttcagtaatgtcttgtttcttttgttgcagtggtgagccattttgacttcgtgaaagtttctttagaatagttgtttccagaggccaaacattccacccgtagtaaagtgcaagcgtaggaagaccaagactggcataaatcaggtataagtgtcgagcactggcaggtgatcttctgaaagtttctactagcagataagatccagtagtcatgcatatggcaacaatgtaccgtgtggatctaagaacgcgtcctactaaccttcgcattcgttggtccagtttgttgttatcgatcaacgtgacaaggttgtcgattccgcgtaagcatgcatacccaaggacgcctgttgcaattccaagtgagccagttccaacaatctttgtaatattagagcacttcattgtgttgcgcttgaaagtaaaatgcgaacaaattaagagataatctcgaaaccgcgacttcaaacgccaatatgatgtgcggcacacaataagcgttcatatccgctgggtgactttctcgctttaaaaaattatccgaaaaaattttctagagtgttgacactttatacttccggctcggataatacgacaaggtgtaaggaggactaaaccatgggtaaggaaaagactcacgt